European Patent Application EP 4 123 022 A1, published January 25, 2023. Title: Protein screening and detection method. Applicant: Universität Zürich. The sequence listing filed with the application follows.

SEQUENCE LISTING (5 sequences)

SEQ ID NO: 1 - protein, 2 aa, Artificial Sequence
  tag sequence
WR

SEQ ID NO: 2 - protein, 3 aa, Artificial Sequence
  tag sequence
WLR

SEQ ID NO: 3 - protein, 4 aa, Artificial Sequence
  tag sequence
WQSR

SEQ ID NO: 4 - protein, 5 aa, Artificial Sequence
  tag sequence
WLTVR

SEQ ID NO: 5 - protein, 6 aa, Artificial Sequence
  tag sequence
WQEGGR